European Patent Application EP 4 119 655 A1, published January 18, 2023. Title: VARIANT OF GENUS YARROWIA AND METHOD OF PREPARING FAT USING THE SAME. Applicant: CJ CheilJedang Corporation. The sequence listing filed with the application follows.

SEQUENCE LISTING (82 sequences)

SEQ ID NO: 1 - DNA, 2829 bp, Yarrowia lipolytica
atggccgttccttctgctgccatcaaggcttccggagtggatatgggggacctcaagaagagacatgacaccaagcttgacgtggaggagagtgtgattgacgagaagatcaatgagaatgaaagcgacgaaaagctgaccgaaaagctgaccgaaaagctgaccgaaaagctgactgaaaagacctccaccgagcccattgcttacgttggcaagtgtcctgatggaacgacttttattgtgccagagacggaggatatgttgaccaacctgtttgatcctcgaatcacaaagtcgctgacggacgtgatcatcgtatcgattctggtcacattcatgggactcttttttgtcgtccccaagtcctggagagtacctctctatctgtttctgtttgccgcatggcgtctggcctacaacggaggaatcggctggctacttcacaaccagtccaactaccacaaactcaccaagtgggctctcaaatacaaggtgtttgacaaggacaacaagacgtggtggcaccagctgattaagcgggagtttgagacccggttccagaaccagcccaactactcgttctacgaggtacccgtcgagttcaacacctggattcttttccgacatgtggtcgatctgattctcatgtcagactttacctgctacttcatgctggcctggtcctgcgctctgtccgtgagaaccaaccagccctggtggcttgttattggacgatggctcgccggagctctaatgctagccttcaacctgtgggctaagactgacgcccaccgagtcgtcaaggattatgcctggtactggggagacttcttcttcctcaaggacatggagttgacttttgatggtgtctttgagatggcccctcatcccatgtactccattggatacgctggtttctacgccgcctctctcatggcctgttcctacaccctgttcctggcctctctggccggccacgctgcccagtttgtgttcctatccatcgttgagaatcctcacattgaaaagacttacaacccccatcagcccaagcagcgacgaaaggcttctcacgtccgagaccgatcttccatccagctggggctcgatcagaaacagaaggatgagctgtctgctattgttgagggcgacgagtccgtttctattgcctctactcccatttctactacttttgacgagccggagactgtccagaaacactcccttcctccgttggttgtgtttagcaacttccagatcactcgagtcacagatatcatgactgtgggagctgcagtctatacaatgctgctctacttcctccctgccaaccgtctgtggtacactgtgacttttttcatggctctgtctgctcgtcttttccacactctgggtcttggagtcatactgcgacgacagtccgagcgacgatccttcaccaagaccttcctcaagtttggaatctacccctttgaggcatacgagcagtggcaagtgtggtacaacgtctccaccgtgttgtcctacaccacatttggtctcttttgcctgcgacagtggagagctccttccaccgatcctctgtggccccttaagtacattcttggcgctctacttattgctctgcatggctggacatcgaagtccatccatgactctcttgggcattttggatggttctacggtgacttcttccttgaccgaaagcagaacctcacttactccggcatttacagatacctcaacaacccagagcgatttttcggtattgctggcatctggggtcttgctctgatgaccaactctccaggtgttggtattttggccttcttgtggactctggagggtatggcattcatcaagttcgtcgagcagccccacatgcagcgaatctacggtaccagtatccgacacgatgctggtgtgaccaagaccattaagaactctctcaagttgccttctccctttgagaaacgggttcgacagttccagggatccgttgacaaggttatcaacgatactctgactgtggtcgaggagttcattggacttgccaagcctactctcaacgaagttgtcaacgactccaagatcctgttgcgacagtaccctgccaaacttacccttactcgaatgctggatgttcccgaaaacattgacactgccgattactctgtgaagctcgtgggcggcgagaagtgtgccgattccaaccgaatttcgtacgcctttggaacccccattcatgtcaagtggcaggcttctcccaacagatcggcaaaggactggatcggtctgtaccgagtgcacgacaacacttcccctgaggtgacttctcttccctccaagggccgatggtctggaatcgacgagactggccatgagtcgcatctcgacggtattgtgtcgtcttctaagaccaatggagaagttgttttccgaggggacacactcttctgggagtgtggagtctacgagttcagataccaccatgctggcaagcacactgtgctcagcacctcggaacctttcgagattgtggctcctaagattgatctatctggagaggtggatgcaaagactctggctcttgagatcctccccatcgtccagcgatgcttctctctatctatggagttccctcctgaggaagtggacgactactgggctcttgaggaacccaaggtgatcaacagagtgcaggctgccgttcaggcgtatttcaacgttgagctggcgcaggaggtgcttcaatcggatgagtctgtggagaatttggctgagcgactgctcagaattagagacgcccttaaaggtcttactgtataa

SEQ ID NO: 2 - protein, 942 aa, Yarrowia lipolytica
MAVPSAAIKASGVDMGDLKKRHDTKLDVEESVIDEKINENESDEKLTEKLTEKLTEKLTEKTSTEPIAYVGKCPDGTTFIVPETEDMLTNLFDPRITKSLTDVIIVSILVTFMGLFFVVPKSWRVPLYLFLFAAWRLAYNGGIGWLLHNQSNYHKLTKWALKYKVFDKDNKTWWHQLIKREFETRFQNQPNYSFYEVPVEFNTWILFRHVVDLILMSDFTCYFMLAWSCALSVRTNQPWWLVIGRWLAGALMLAFNLWAKTDAHRVVKDYAWYWGDFFFLKDMELTFDGVFEMAPHPMYSIGYAGFYAASLMACSYTLFLASLAGHAAQFVFLSIVENPHIEKTYNPHQPKQRRKASHVRDRSSIQLGLDQKQKDELSAIVEGDESVSIASTPISTTFDEPETVQKHSLPPLVVFSNFQITRVTDIMTVGAAVYTMLLYFLPANRLWYTVTFFMALSARLFHTLGLGVILRRQSERRSFTKTFLKFGIYPFEAYEQWQVWYNVSTVLSYTTFGLFCLRQWRAPSTDPLWPLKYILGALLIALHGWTSKSIHDSLGHFGWFYGDFFLDRKQNLTYSGIYRYLNNPERFFGIAGIWGLALMTNSPGVGILAFLWTLEGMAFIKFVEQPHMQRIYGTSIRHDAGVTKTIKNSLKLPSPFEKRVRQFQGSVDKVINDTLTVVEEFIGLAKPTLNEVVNDSKILLRQYPAKLTLTRMLDVPENIDTADYSVKLVGGEKCADSNRISYAFGTPIHVKWQASPNRSAKDWIGLYRVHDNTSPEVTSLPSKGRWSGIDETGHESHLDGIVSSSKTNGEVVFRGDTLFWECGVYEFRYHHAGKHTVLSTSEPFEIVAPKIDLSGEVDAKTLALEILPIVQRCFSLSMEFPPEEVDDYWALEEPKVINRVQAAVQAYFNVELAQEVLQSDESVENLAERLLRIRDALKGLTV

SEQ ID NO: 3 - DNA, 40 bp, Artificial Sequence
  CHO2_5_For
gtacccggggatcctctagagtcatccgcaaacacaacac

SEQ ID NO: 4 - DNA, 40 bp, Artificial Sequence
  CHO2_5_Rev
gcaatgacgagtcagacaggggtgtttgtggaagctggtg

SEQ ID NO: 5 - DNA, 40 bp, Artificial Sequence
  CHO2_URA_For
caccagcttccacaaacacccctgtctgactcgtcattgc

SEQ ID NO: 6 - DNA, 40 bp, Artificial Sequence
  CHO2_URA_Rev
cgcattctgcgtacattttgctggtggtattgtgactggg

SEQ ID NO: 7 - DNA, 40 bp, Artificial Sequence
  CHO2_5RP_For
cccagtcacaataccaccagcaaaatgtacgcagaatgcg

SEQ ID NO: 8 - DNA, 40 bp, Artificial Sequence
  CHO2_5RP_Rev
cagatatgctctctgcaaacggtgtttgtggaagctggtg

SEQ ID NO: 9 - DNA, 40 bp, Artificial Sequence
  CHO2_3_For
caccagcttccacaaacaccgtttgcagagagcatatctg

SEQ ID NO: 10 - DNA, 40 bp, Artificial Sequence
  CHO2_3_Rev
gcaggtcgactctagagagaggtctgttcacaacatcggc

SEQ ID NO: 11 - DNA, 627 bp, Yarrowia lipolytica
atgtcctttcctgacaagattgttgccgacttcaacgtggattacgaccagaagagcctctggatcgtcctgggctccatcgccttcaaccccatcttttggaacattgttgctcgagccgagtacaacacccactttctgactaagctggctggaggagccaagaccggatgctatctgctggccatcaccattttctcgctcggtatcttccgagactacctttaccaccaggctcttgagcagcagcccacctccattctgctgtcggtcacttacgttgacattgtcaagcctctggccattgtgctgtttgctgttggcaacgtgctggtccttacctccatgtacgccctgggcgtcaccggaacctacctcggcgactactttggcattctcatgaacgagcgagtcaccggcttccccttcaatgtgtccaacaaccccatgtaccacggctccactctgtgtttcctggcttccgctctgtggtacgccaagcccgcaggcctgctcatcaccgcctttgtgtcgctcatgtactccattgctctcaagttcgaggaacccttcaccggtgagatctacgctaagcgagaccgggagctcgctgccaagcagaagtaa

SEQ ID NO: 12 - protein, 208 aa, Yarrowia lipolytica
MSFPDKIVADFNVDYDQKSLWIVLGSIAFNPIFWNIVARAEYNTHFLTKLAGGAKTGCYLLAITIFSLGIFRDYLYHQALEQQPTSILLSVTYVDIVKPLAIVLFAVGNVLVLTSMYALGVTGTYLGDYFGILMNERVTGFPFNVSNNPMYHGSTLCFLASALWYAKPAGLLITAFVSLMYSIALKFEEPFTGEIYAKRDRELAAKQK

SEQ ID NO: 13 - DNA, 40 bp, Artificial Sequence
  OPI3_5_For
gtacccggggatcctctagacaccaacattcgacatggac

SEQ ID NO: 14 - DNA, 40 bp, Artificial Sequence
  OPI3_5_Rev
gcaatgacgagtcagacagggagttttccagagagccaac

SEQ ID NO: 15 - DNA, 40 bp, Artificial Sequence
  OPI3_URA_For
gttggctctctggaaaactccctgtctgactcgtcattgc

SEQ ID NO: 16 - DNA, 40 bp, Artificial Sequence
  OPI3_URA_Rev
cagtccttaatcaacggtggctggtggtattgtgactggg

SEQ ID NO: 17 - DNA, 40 bp, Artificial Sequence
  OPI3_5RP_For
cccagtcacaataccaccagccaccgttgattaaggactg

SEQ ID NO: 18 - DNA, 40 bp, Artificial Sequence
  OPI3_5RP_Rev
cgtaggccgttttctgttgcgagttttccagagagccaac

SEQ ID NO: 19 - DNA, 40 bp, Artificial Sequence
  OPI3_3_For
gttggctctctggaaaactcgcaacagaaaacggcctacg

SEQ ID NO: 20 - DNA, 40 bp, Artificial Sequence
  OPI3_3_Rev
gcaggtcgactctagagagtgccgtctcgattgtcacagg

SEQ ID NO: 21 - DNA, 2103 bp, Yarrowia lipolytica
atgaaccccaacaacactggcaccattgaaatcaacggtaaggagtacaacaccttcaccgagccccccgtggccatggctcaggagcgagccaagacctccttccccgtgcgagagatgacctacttcctcgacggtggcgagaagaacaccctcaaaaacgagcagatcatggaggagattgagcgagaccctcttttcaacaacgacaactactacgatctcaacaaggagcagatccgagagctcaccatggagcgagtcgccaagctgtctctgtttgtgcgtgatcagcccgaggacgacatcaagaagcgatttgctctcattggtatcgccgatatgggaacctacacccgacttggtgtccactacggcctcttctttggcgccgtccgaggtaccggaactgccgagcagtttggccactggatctccaagggagccggagacctgcgaaagttctacggatgtttctccatgaccgagctgggccatggctccaacctggctggtctcgagaccaccgccatctacgatgaggagaccgacgagttcatcatcaacacccctcacattgccgccaccaagtggtggattggaggagccgcccacaccgccacccacactgtcgtgttcgcccgactcattgtcaagggcaaggactacggtgtcaagacctttgttgtccagctgcgaaacatcaacgaccacagcctcaaggtcggtatctctattggtgatatcggaaagaagatgggccgagacggtatcgataacggatggatccagttcaccaacgtgcgaatcccccgacagaacctgctcatgaagtacacaaaggtcgaccgagagggtaacgtgacccagcctcctctggctcagcttacctacggttctcttatcactggtcgagtctccatggcctctgattctcaccaggtcggaaagcgattcatcaccattgctctgcgatacgcctgcattcgacgacagttctccaccacccccggccagcccgagaccaagatcatcgactacccctaccatcagcgacgacttctgcctcttctggcctatgtctatgctcttaagatgactgccgatgaggttggagctctcttctcccgaaccatgcttaagatggacgacctcaagcccgacgacaaggccggcctcaatgaggttgtttccgacgtcaaggagctcttctccgtctccgccggtctcaaggccttctccacctgggcttgtgccgacgtcattgacaagacccgacaggcttgcggtggccacggttactctggatacaacggtttcggccaggcctacgccgactgggttgtccagtgcacctgggagggtgacaacaacattctcaccctttctgccggccgagctcttatccagtctgccgttgctctgcgaaagggcgagcctgttggtaacgccgtttcttacctgaagcgatacaaggatctggccaacgctaagctcaatggccgatctctcaccgaccccaaggtcctcgtcgaggcctgggaggttgctgccggtaacatcatcaaccgagccaccgaccagtacgagaagctcattggcgagggtcttaacgccgaccaggcctttgaggttctgtctcagcagcgattccaggccgccaaggtccacacacgacgacacctcattgccgctttcttctcccgaattgacaccgaggctggcgaggccatcaagcagcccctgcttaacctggctctgctgtttgccctgtggtccatcgaagaggactctggtctgttcctgcgagagggcttcctcgagcccaaggatatcgacaccgtcaccgagctcgtcaacaagtactgcaccactgtgcgagaggaggtcattggctacaccgatgccttcaacctgtccgactacttcatcaacgctcctattggatgctacgatggtgacgcttaccgacactacttccagaaggtcaacgagcagaaccctgcccgagacccccgacctccttactacgcctctactctcaagcccttccttttccgagaggaggaggatgatgacatttgcgagcttgatgaggaatag

SEQ ID NO: 22 - protein, 700 aa, Yarrowia lipolytica
MNPNNTGTIEINGKEYNTFTEPPVAMAQERAKTSFPVREMTYFLDGGEKNTLKNEQIMEEIERDPLFNNDNYYDLNKEQIRELTMERVAKLSLFVRDQPEDDIKKRFALIGIADMGTYTRLGVHYGLFFGAVRGTGTAEQFGHWISKGAGDLRKFYGCFSMTELGHGSNLAGLETTAIYDEETDEFIINTPHIAATKWWIGGAAHTATHTVVFARLIVKGKDYGVKTFVVQLRNINDHSLKVGISIGDIGKKMGRDGIDNGWIQFTNVRIPRQNLLMKYTKVDREGNVTQPPLAQLTYGSLITGRVSMASDSHQVGKRFITIALRYACIRRQFSTTPGQPETKIIDYPYHQRRLLPLLAYVYALKMTADEVGALFSRTMLKMDDLKPDDKAGLNEVVSDVKELFSVSAGLKAFSTWACADVIDKTRQACGGHGYSGYNGFGQAYADWVVQCTWEGDNNILTLSAGRALIQSAVALRKGEPVGNAVSYLKRYKDLANAKLNGRSLTDPKVLVEAWEVAAGNIINRATDQYEKLIGEGLNADQAFEVLSQQRFQAAKVHTRRHLIAAFFSRIDTEAGEAIKQPLLNLALLFALWSIEEDSGLFLREGFLEPKDIDTVTELVNKYCTTVREEVIGYTDAFNLSDYFINAPIGCYDGDAYRHYFQKVNEQNPARDPRPPYYASTLKPFLFREEEDDDICELDEE

SEQ ID NO: 23 - DNA, 2706 bp, Yarrowia lipolytica
atgtctggagaactaagatacgacggaaaggtcgtcattgttaccggtgccggtggcggtctcggtaaggcatacgcccttttctacggctctcgaggagcctctgttgttgtcaacgatcttggtggcgacttcaagggcgacggtgcccaggctggcagtggcaagcgagttgccgatgttgtcgtcgacgagattgtttccaagggaggcaaggctgttgctaactacgactctgtcgagaacggtgacaagattgtcgagactgccgtcaaggcttttggctccgtccacattgtcatcaacaacgccggtattctccgagatatttccttcaagaagatgaccgacaaggactgggatcttgtctacaaggtccacgttttcggtgcctacaaggttacccgagctgcctggccttacttccgaaagcagaagtacggtcgagttatctctacctcttccgctgctggtctttacggaaacttcggccagaccaactactccgctgccaagctcgccctggttggtttcggtgagactctcgccaaggagggtgccaagtacaacattacttccaacgtcatcgctcctcttgctgcttcccgaatgaccgagacagtcatgcccgaggatatcctcaagctcctcaagcctgagtacgttgttcctctggtcggctacctcacccacgactctgtcaccgagtcttatggtatttacgaggtcggtgctggttacatggctaaaatccgatgggagcgaggcaacggtgctgttttcaagggcgacgacactttcaccccgtctgctattctgaagcgatgggatgaggtcacctcttttgagagccccacctaccctaacggccctgctgacttcttcaaatacgctgaggagtctgttaagcgacccgagaacccccagggacccaccgtctccttcaaggaccaggttgtcattgtcactggagccggtgctggcattggccgagcttactctcacctccttgctaagcttggtgccaaggtcgttgttaacgatttcggtaaccctcagaaggttgtcgatgaaattaaggccctcggtggtatcgccgtcgctgacaagaacaacgtcatccacggtgagaaggttgttcagaccgctatcgacgccttcggtgctgtccacgccgttgtcaacaacgctggtattctccgagacaagtctttcgccaacatggatgatgagatgtggcagctgatctttgatgtccacctcaacggtacttactccgttaccaaggccgcgtggccccacttccttaagcagaagtacggccgtgtcatcaacaccacctcaacttctggtatctacggtaacttcggccaggccaactactctgccgccaaggctggtatcctcggtttctcccgagctcttgctcgagagggtgagaagtacaacattcttgtcaacaccattgcccctaacgctggtactgccatgactgcttctgtcttcactgaggagatgctcgagctcttcaagcccgatttcatcgcacccatcaccgtcctgcttgcttccgatcaggctcccgtcaccggtgatctgtttgagactggttctgcttggatcggacagactcgatggcagcgagctggtggtaaggccttcaacaccaagaagggtgtcacccccgaaatggttcgagacagctgggctaagatcgtcgacttcgatgatggtaactccacccatcccaccactccctccgagtctactactcagattcttgagaacatcttcaacgtgcctgatgaggaggttgaggagactgctctcgttgctggtcccggtggtcccggtatcctcaacaaggagggcgaacctttcgactacacttacacttaccgagacctcattctttacaaccttggtctcggtgccaaggctaatgagctcaagtatgtcttcgagggtgatgatgacttccagaccgtgcccactttcggtgttatcccttacatgggtggcctcatcactaccaactatggcgacttcgttcctaacttcaaccctatgatgcttctccacggtgagcagtaccttgaaatccgacagtggcctattcctaccaatgctacattggagaacaaggctaaggtcatcgatgtcgttgacaagggcaaggctgccctccttgtcactgctaccaccaccacgaacaaggagactggtgaggaggttttctacaacgagtcttctctcttcatccgaggctctggtggtttcggtggtaagtctaccggtactgaccgtggcgctgccactgctgccaacaagccccctgctcgagctcctgacttcgttaaggagatcaagatccaggaggaccaggctgccatttaccgactttctggtgattacaaccctcttcacatcgaccctgcttttgctgctgttggtaactttgaccgacctattctccacggtctctgctcttttggtgtctccggtaaggctctttacgatcagtttggtcctttcaagaacgctaaggtccgatttgctggtcacgtcttccctggtgagaccctgaaggttgagggctggaaggagggcaacaaggtcattttccagaccaaggttgttgagcgaggtactaccgccatcagcaatgccgccattgagctcttccccaaggatgctaagctctaa

SEQ ID NO: 24 - protein, 901 aa, Yarrowia lipolytica
MSGELRYDGKVVIVTGAGGGLGKAYALFYGSRGASVVVNDLGGDFKGDGAQAGSGKRVADVVVDEIVSKGGKAVANYDSVENGDKIVETAVKAFGSVHIVINNAGILRDISFKKMTDKDWDLVYKVHVFGAYKVTRAAWPYFRKQKYGRVISTSSAAGLYGNFGQTNYSAAKLALVGFGETLAKEGAKYNITSNVIAPLAASRMTETVMPEDILKLLKPEYVVPLVGYLTHDSVTESYGIYEVGAGYMAKIRWERGNGAVFKGDDTFTPSAILKRWDEVTSFESPTYPNGPADFFKYAEESVKRPENPQGPTVSFKDQVVIVTGAGAGIGRAYSHLLAKLGAKVVVNDFGNPQKVVDEIKALGGIAVADKNNVIHGEKVVQTAIDAFGAVHAVVNNAGILRDKSFANMDDEMWQLIFDVHLNGTYSVTKAAWPHFLKQKYGRVINTTSTSGIYGNFGQANYSAAKAGILGFSRALAREGEKYNILVNTIAPNAGTAMTASVFTEEMLELFKPDFIAPITVLLASDQAPVTGDLFETGSAWIGQTRWQRAGGKAFNTKKGVTPEMVRDSWAKIVDFDDGNSTHPTTPSESTTQILENIFNVPDEEVEETALVAGPGGPGILNKEGEPFDYTYTYRDLILYNLGLGAKANELKYVFEGDDDFQTVPTFGVIPYMGGLITTNYGDFVPNFNPMMLLHGEQYLEIRQWPIPTNATLENKAKVIDVVDKGKAALLVTATTTTNKETGEEVFYNESSLFIRGSGGFGGKSTGTDRGAATAANKPPARAPDFVKEIKIQEDQAAIYRLSGDYNPLHIDPAFAAVGNFDRPILHGLCSFGVSGKALYDQFGPFKNAKVRFAGHVFPGETLKVEGWKEGNKVIFQTKVVERGTTAISNAAIELFPKDAKL

SEQ ID NO: 25 - DNA, 1134 bp, Yarrowia lipolytica
atgtggggaagttcacatgcattcgctggtgaatctgatctgacactacaactacacaccaggtccaacatgagcgacaatacgacaatcaaaaagccgatccgacccaaaccgatccggacggaacgcctgccttacgctggggccgcagaaatcatccgagccaaccagaaagaccactactttgagtccgtgcttgaacagcatctcgtcacgtttctgcagaaatggaagggagtacgatttatccaccagtacaaggaggagctggagacggcgtccaagtttgcatatctcggtttgtgtacgcttgtgggctccaagactctcggagaagagtacaccaatctcatgtacactatcagagaccgaacagctctaccgggggtggtgagacggtttggctacgtgctttccaacactctgtttccatacctgtttgtgcgctacatgggcaagttgcgcgccaaactgatgcgcgagtatccccatctggtggagtacgacgaagatgagcctgtgcccagcccggaaacatggaaggagcgggtcatcaagacgtttgtgaacaagtttgacaagttcacggcgctggaggggtttaccgcgatccacttggcgattttctacgtctacggctcgtactaccagctcagtaagcggatctggggcatgcgttatgtatttggacaccgactggacaagaatgagcctcgaatcggttacgagatgctcggtctgctgattttcgcccggtttgccacgtcatttgtgcagacgggaagagagtacctcggagcgctgctggaaaagagcgtggagaaagaggcaggggagaaggaagatgaaaaggaagcggttgtgccgaaaaagaagtcgtcaattccgttcattgaggatacagaaggggagacggaagacaagatcgatctggaggaccctcgacagctcaagttcattcctgaggcgtccagagcgtgcactctgtgtctgtcatacattagtgcgccggcatgtacgccatgtggacactttttctgttgggactgtatttccgaatgggtgagagagaagcccgagtgtcccttgtgtcggcagggtgtgagagagcagaacttgttgcctatcagataa

SEQ ID NO: 26 - protein, 377 aa, Yarrowia lipolytica
MWGSSHAFAGESDLTLQLHTRSNMSDNTTIKKPIRPKPIRTERLPYAGAAEIIRANQKDHYFESVLEQHLVTFLQKWKGVRFIHQYKEELETASKFAYLGLCTLVGSKTLGEEYTNLMYTIRDRTALPGVVRRFGYVLSNTLFPYLFVRYMGKLRAKLMREYPHLVEYDEDEPVPSPETWKERVIKTFVNKFDKFTALEGFTAIHLAIFYVYGSYYQLSKRIWGMRYVFGHRLDKNEPRIGYEMLGLLIFARFATSFVQTGREYLGALLEKSVEKEAGEKEDEKEAVVPKKKSSIPFIEDTEGETEDKIDLEDPRQLKFIPEASRACTLCLSYISAPACTPCGHFFCWDCISEWVREKPECPLCRQGVREQNLLPIR

SEQ ID NO: 27 - DNA, 1245 bp, Yarrowia lipolytica
atggaccgacttaacaacctcgccacccagctcgagcagaaccccgccaagggcctcgacgctatcacctccaagaaccccgatgacgttgtcatcaccgccgcctaccgaactgcccacaccaagggaggcaagggtctgttcaaggacacctcttcttccgagctgctcgcctctctgctggagggcctcgtcaaggagtccaagatcgaccccaagctcatcggtgatgtcgtctgcgggaacgttctcgctgccggtgccggtgccactgagcaccgagctgcctgccttgttgccggcatccccgagaccgttcccttcgtcgctctcaaccgacagtgctcctctggtctgatggccgtcaacgacgttgccaacaagatccgagccggccagattgacattggtatcggctgtggtgtcgagtccatgtccaaccagtacggtcccaactccgtcacccccttctccaacaagttccagaacaacgaggaggctaagaagtgcctgatccccatgggtatcacttccgagaacgttgccgccaagtacaacgtgtcccgaaaggcccaggacgcctttgctgccaagtcctacgagaaggccgccgctgcccaggccgccggcaagttcgaccaggagatcctccccatcaagaccactgttctcgatgatgatgacaacgagaaggaggttaccgtcaacaaggacgacggtatccgacctggtgtcaccgccgagaagctcggcaagctcaagcctgctttctccgccgagggaaccacccacgctggtaacgcctctcagatctccgacggtgccggagccgttctcctcatgcgacgatctgttgccgagaagcttggccagcccatccttgccaagtttgtccactgcaagaccgtcggtgttccccccgagctcatgggaattggccccgcttacgccattcctgctgtccttgaggaccttggtctgaccgtcaacgacgttgacgttttcgagatcaacgaggctttcgcttcccaggctctgttctccatccagcattgtggaatcgacgagtccaaggtcaacccccgaggtggtgccattgctattggccaccctctgggagccaccggtgctcgacagtttgccactctgctctccgagcttaaggagtctggcaagaaggtcggtgtcacctccatgtgcattggtaccggtatgggtgccgcttctctggttgttgccgagtaa

SEQ ID NO: 28 - protein, 414 aa, Yarrowia lipolytica
MDRLNNLATQLEQNPAKGLDAITSKNPDDVVITAAYRTAHTKGGKGLFKDTSSSELLASLLEGLVKESKIDPKLIGDVVCGNVLAAGAGATEHRAACLVAGIPETVPFVALNRQCSSGLMAVNDVANKIRAGQIDIGIGCGVESMSNQYGPNSVTPFSNKFQNNEEAKKCLIPMGITSENVAAKYNVSRKAQDAFAAKSYEKAAAAQAAGKFDQEILPIKTTVLDDDDNEKEVTVNKDDGIRPGVTAEKLGKLKPAFSAEGTTHAGNASQISDGAGAVLLMRRSVAEKLGQPILAKFVHCKTVGVPPELMGIGPAYAIPAVLEDLGLTVNDVDVFEINEAFASQALFSIQHCGIDESKVNPRGGAIAIGHPLGATGARQFATLLSELKESGKKVGVTSMCIGTGMGAASLVVAE

SEQ ID NO: 29 - DNA, 858 bp, Yarrowia lipolytica
atggacctcgaattggaaattcccgtcttgcattccatggactcgcaccaccaggtggtggactcccacagactggcacagcaacagttccagtaccagcagatccacatgctgcagcagacgctgtcacagcagtacccccacaccccatccaccacaccccccatttacatgctgtcgcctgcggactacgagaaggacgccgtttccatctcaccggtaatgctgtggcccccctcggcccactcccaggcctcttaccattacgagatgccctccgttatctcgccatctccttctcccactagatccttctgtaatccgagagagctggaggttcaggacgagctcgagcagcttgaacagcagcccgccgctctctccgtcgaacatctgtttgacattgagaactcatcgatcgagtatgcacacgacgagctgcatgacacctcttcgtgctccgactcgcagtcgagcttttcccctcagcagtcccctgcctccccggcctccacttactcgcctctcgaggacgagtttctcaacttggctggatccgagttgaagagcgagcccagcgcggacgacgagaaggatgatgtggacacggagcttccccagcagcccgagatcatcatccctgtgtcgtgccgaggccgaaagccgtccatcgacgactccaaaaagacttttgtctgcacccactgccagcgtcggttccggcgccaggagcatctcaagcgacatttccgatccctacacactcgagagaagcctttcaactgcgacacgtgcggcaagaagttttctcggtcggacaatctcgcccagcatatgcgtacgcatcctcgggactag

SEQ ID NO: 30 - protein, 285 aa, Yarrowia lipolytica
MDLELEIPVLHSMDSHHQVVDSHRLAQQQFQYQQIHMLQQTLSQQYPHTPSTTPPIYMLSPADYEKDAVSISPVMLWPPSAHSQASYHYEMPSVISPSPSPTRSFCNPRELEVQDELEQLEQQPAALSVEHLFDIENSSIEYAHDELHDTSSCSDSQSSFSPQQSPASPASTYSPLEDEFLNLAGSELKSEPSADDEKDDVDTELPQQPEIIIPVSCRGRKPSIDDSKKTFVCTHCQRRFRRQEHLKRHFRSLHTREKPFNCDTCGKKFSRSDNLAQHMRTHPRD

SEQ ID NO: 31 - DNA, 40 bp, Artificial Sequence
  POX2_5_For
gtacccggggatcctctagagattccgccaagtgagactg

SEQ ID NO: 32 - DNA, 40 bp, Artificial Sequence
  POX2_5_Rev
gcaatgacgagtcagacaggcgttgcttgtgtgatttttg

SEQ ID NO: 33 - DNA, 40 bp, Artificial Sequence
  POX2_URA_For
caaaaatcacacaagcaacgcctgtctgactcgtcattgc

SEQ ID NO: 34 - DNA, 40 bp, Artificial Sequence
  POX2_URA_Rev
cgcttgtccagtatgaatagctggtggtattgtgactggg

SEQ ID NO: 35 - DNA, 40 bp, Artificial Sequence
  POX2_5RP_For
cccagtcacaataccaccagctattcatactggacaagcg

SEQ ID NO: 36 - DNA, 39 bp, Artificial Sequence
  POX2_5RP_Rev
caataaatacccgcttgtccgttgcttgtgtgatttttg

SEQ ID NO: 37 - DNA, 39 bp, Artificial Sequence
  POX2_3_For
caaaaatcacacaagcaacggacaagcgggtatttattg

SEQ ID NO: 38 - DNA, 36 bp, Artificial Sequence
  POX2_3_Rev
gcaggtcgactctagaccaaacaaagctgatgacac

SEQ ID NO: 39 - DNA, 40 bp, Artificial Sequence
  MFE1_5_For
gtacccggggatcctctagacaagccaaagagatgttgac

SEQ ID NO: 40 - DNA, 40 bp, Artificial Sequence
  MFE1_5_Rev
gcaatgacgagtcagacagggttaataacgtatcttctac

SEQ ID NO: 41 - DNA, 40 bp, Artificial Sequence
  MFE1_URA_For
gtagaagatacgttattaaccctgtctgactcgtcattgc

SEQ ID NO: 42 - DNA, 40 bp, Artificial Sequence
  MFE1_URA_Rev
caaatcagccgttggcctgcctggtggtattgtgactggg

SEQ ID NO: 43 - DNA, 40 bp, Artificial Sequence
  MFE1_5RP_For
cccagtcacaataccaccaggcaggccaacggctgatttg

SEQ ID NO: 44 - DNA, 39 bp, Artificial Sequence
  MFE1_5RP_Rev
cacttggtcagataatagcgttaataacgtatcttctac

SEQ ID NO: 45 - DNA, 39 bp, Artificial Sequence
  MFE1_3_For
gtagaagatacgttattaacgctattatctgaccaagtg

SEQ ID NO: 46 - DNA, 38 bp, Artificial Sequence
  MFE1_3_Rev
gcaggtcgactctagatgcttgaaggcatatgtgactg

SEQ ID NO: 47 - DNA, 40 bp, Artificial Sequence
  PEX10_5_For
gtacccggggatcctctagagttttcgtcttagcgtcatg

SEQ ID NO: 48 - DNA, 40 bp, Artificial Sequence
  PEX10_5_Rev
gcaatgacgagtcagacagggccgaggcagatttgggttg

SEQ ID NO: 49 - DNA, 40 bp, Artificial Sequence
  PEX10_URA_For
caacccaaatctgcctcggccctgtctgactcgtcattgc

SEQ ID NO: 50 - DNA, 40 bp, Artificial Sequence
  PEX10_URA_Rev
gagtccagtaattctttccgctggtggtattgtgactggg

SEQ ID NO: 51 - DNA, 40 bp, Artificial Sequence
  PEX10_5RP_For
cccagtcacaataccaccagcggaaagaattactggactc

SEQ ID NO: 52 - DNA, 40 bp, Artificial Sequence
  PEX10_5RP_Rev
ccttccatccagacctcgtcgccgaggcagatttgggttg

SEQ ID NO: 53 - DNA, 40 bp, Artificial Sequence
  PEX10_3_For
caacccaaatctgcctcggcgacgaggtctggatggaagg

SEQ ID NO: 54 - DNA, 40 bp, Artificial Sequence
  PEX10_3_Rev
gcaggtcgactctagagctgacctataccagatcagacgc

SEQ ID NO: 55 - DNA, 40 bp, Artificial Sequence
  POT1_5_For
gtacccggggatcctctagacacaataccccacagtgtgc

SEQ ID NO: 56 - DNA, 40 bp, Artificial Sequence
  POT1_5_Rev
gcaatgacgagtcagacagggtgtgtcttggttggatgag

SEQ ID NO: 57 - DNA, 40 bp, Artificial Sequence
  POT1_URA_For
ctcatccaaccaagacacaccctgtctgactcgtcattgc

SEQ ID NO: 58 - DNA, 40 bp, Artificial Sequence
  POT1_URA_Rev
caggcgctcccccattggcgctggtggtattgtgactggg

SEQ ID NO: 59 - DNA, 40 bp, Artificial Sequence
  POT1_5RP_For
cccagtcacaataccaccagcgccaatgggggagcgcctg

SEQ ID NO: 60 - DNA, 40 bp, Artificial Sequence
  POT1_5RP_Rev
gttcgatcgcgattcatttcgtgtgtcttggttggatgag

SEQ ID NO: 61 - DNA, 40 bp, Artificial Sequence
  POT1_3_For
ctcatccaaccaagacacacgaaatgaatcgcgatcgaac

SEQ ID NO: 62 - DNA, 40 bp, Artificial Sequence
  POT1_3_Rev
gcaggtcgactctagagaggagtgctaaaattagccctgc

SEQ ID NO: 63 - DNA, 39 bp, Artificial Sequence
  MHY1_5_For
gtacccggggatcctctagatgtcagcgaaagctcaaag

SEQ ID NO: 64 - DNA, 40 bp, Artificial Sequence
  MHY1_5_Rev
gcaatgacgagtcagacaggcaattcgaggtccattttgg

SEQ ID NO: 65 - DNA, 40 bp, Artificial Sequence
  MHY1_URA_For
ccaaaatggacctcgaattgcctgtctgactcgtcattgc

SEQ ID NO: 66 - DNA, 40 bp, Artificial Sequence
  MHY1_URA_Rev
gtggtgcttttgtacttgtcctggtggtattgtgactggg

SEQ ID NO: 67 - DNA, 40 bp, Artificial Sequence
  MHY1_5RP_For
cccagtcacaataccaccaggacaagtacaaaagcaccac

SEQ ID NO: 68 - DNA, 40 bp, Artificial Sequence
  MHY1_5RP_Rev
gaaggcgctctacctctagtccaattcgaggtccattttg

SEQ ID NO: 69 - DNA, 40 bp, Artificial Sequence
  MHY1_3_For
caaaatggacctcgaattggactagaggtagagcgccttc

SEQ ID NO: 70 - DNA, 40 bp, Artificial Sequence
  MHY1_3_Rev
gcaggtcgactctagactgtgtttgattagctcttctcag

SEQ ID NO: 71 - DNA, 1545 bp, Yarrowia lipolytica
atgactatcgactcacaatactacaagtcgcgagacaaaaacgacacggcacccaaaatcgcgggaatccgatatgccccgctatcgacaccattactcaaccgatgtgagaccttctctctggtctggcacattttcagcattcccactttcctcacaattttcatgctatgctgcgcaattccactgctctggccatttgtgattgcgtatgtagtgtacgctgttaaagacgactccccgtccaacggaggagtggtcaagcgatactcgcctatttcaagaaacttcttcatctggaagctctttggccgctacttccccataactctgcacaagacggtggatctggagcccacgcacacatactaccctctggacgtccaggagtatcacctgattgctgagagatactggccgcagaacaagtacctccgagcaatcatctccaccatcgagtactttctgcccgccttcatgaaacggtctctttctatcaacgagcaggagcagcctgccgagcgagatcctctcctgtctcccgtttctcccagctctccgggttctcaacctgacaagtggattaaccacgacagcagatatagccgtggagaatcatctggctccaacggccacgcctcgggctccgaacttaacggcaacggcaacaatggcaccactaaccgacgacctttgtcgtccgcctctgctggctccactgcatctgattccacgcttcttaacgggtccctcaactcctacgccaaccagatcattggcgaaaacgacccacagctgtcgcccacaaaactcaagcccactggcagaaaatacatcttcggctaccacccccacggcattatcggcatgggagcctttggtggaattgccaccgagggagctggatggtccaagctctttccgggcatccctgtttctcttatgactctcaccaacaacttccgagtgcctctctacagagagtacctcatgagtctgggagtcgcttctgtctccaagaagtcctgcaaggccctcctcaagcgaaaccagtctatctgcattgtcgttggtggagcacaggaaagtcttctggccagacccggtgtcatggacctggtgctactcaagcgaaagggttttgttcgacttggtatggaggtcggaaatgtcgcccttgttcccatcatggcctttggtgagaacgacctctatgaccaggttagcaacgacaagtcgtccaagctgtaccgattccagcagtttgtcaagaacttccttggattcacccttcctttgatgcatgcccgaggcgtcttcaactacgatgtcggtcttgtcccctacaggcgacccgtcaacattgtggttggttcccccattgacttgccttatctcccacaccccaccgacgaagaagtgtccgaataccacgaccgatacatcgccgagctgcagcgaatctacaacgagcacaaggatgaatatttcatcgattggaccgaggagggcaaaggagccccagagttccgaatgattgagtaa

SEQ ID NO: 72 - protein, 514 aa, Yarrowia lipolytica
MTIDSQYYKSRDKNDTAPKIAGIRYAPLSTPLLNRCETFSLVWHIFSIPTFLTIFMLCCAIPLLWPFVIAYVVYAVKDDSPSNGGVVKRYSPISRNFFIWKLFGRYFPITLHKTVDLEPTHTYYPLDVQEYHLIAERYWPQNKYLRAIISTIEYFLPAFMKRSLSINEQEQPAERDPLLSPVSPSSPGSQPDKWINHDSRYSRGESSGSNGHASGSELNGNGNNGTTNRRPLSSASAGSTASDSTLLNGSLNSYANQIIGENDPQLSPTKLKPTGRKYIFGYHPHGIIGMGAFGGIATEGAGWSKLFPGIPVSLMTLTNNFRVPLYREYLMSLGVASVSKKSCKALLKRNQSICIVVGGAQESLLARPGVMDLVLLKRKGFVRLGMEVGNVALVPIMAFGENDLYDQVSNDKSSKLYRFQQFVKNFLGFTLPLMHARGVFNYDVGLVPYRRPVNIVVGSPIDLPYLPHPTDEEVSEYHDRYIAELQRIYNEHKDEYFIDWTEEGKGAPEFRMIE

SEQ ID NO: 73 - DNA, 40 bp, Artificial Sequence
  DGA1_5_For
gtacccggggatcctctagagacgagaaacaaatcatgtg

SEQ ID NO: 74 - DNA, 41 bp, Artificial Sequence
  DGA1_5_Rev
cgccgccaacccggtctctagcttttgttttgtgtgacttg

SEQ ID NO: 75 - DNA, 41 bp, Artificial Sequence
  DGA1_TEF1_For
caagtcacacaaaacaaaagctagagaccgggttggcggcg

SEQ ID NO: 76 - DNA, 42 bp, Artificial Sequence
  DGA1_TEF1_Rev
gacgagtcagacaggaggcactgcggttagtactgcaaaaag

SEQ ID NO: 77 - DNA, 42 bp, Artificial Sequence
  DGA1_URA_For
ctttttgcagtactaaccgcagtgcctcctgtctgactcgtc

SEQ ID NO: 78 - DNA, 38 bp, Artificial Sequence
  DGA1_URA_Rev
cgccgccaacccggtctcttggtggtattgtgactggg

SEQ ID NO: 79 - DNA, 38 bp, Artificial Sequence
  DGA1_TEF2_For
cccagtcacaataccaccaagagaccgggttggcggcg

SEQ ID NO: 80 - DNA, 43 bp, Artificial Sequence
  DGA1_TEF2_Rev
gtagtattgtgagtcgatagtctgcggttagtactgcaaaaag

SEQ ID NO: 81 - DNA, 43 bp, Artificial Sequence
  DGA1_dga1_For
ctttttgcagtactaaccgcagactatcgactcacaatactac

SEQ ID NO: 82 - DNA, 41 bp, Artificial Sequence
  DGA1_dga1_Rev
gcctgcaggtcgactctagattactcaatcattcggaactc